European Patent Application EP 4 772 619 A1, published July 8, 2026. Title: 嘧啶核苷磷酸化酶突变体及2'-氟代核苷的制备方法. Applicant: 吉林凯莱英制药有限公司. The sequence listing filed with the application follows.

SEQUENCE LISTING (3 sequences)

SEQ ID NO: 1 - protein, 423 aa, Thermus thermophilus
MNPVAFIREKREGKKHRREDLEAFLLGYLHDEVPDYQVSAWLMAAFLRGLDPEETLWLTETMARSGKVLDLSGLPHPVDQHSSGGVGDKVSLVVGPILAASGCTFAKMSGRTLAHTGGNIDKLESVPGWRGEMTEAEFLERARRVGLVIAAQSPDLTPLDGKLYALRDVTATTESVPLIASSIMSKKLAVGARSIVLDVKVGRGAFMKTLEEARLLAKTMVAIGQGDGRRVRALLTSMEAPLGRAVGNAIEVREAIEALKGEGPGDLLEVALALAEEALRREGLDPALARKALEGGAALEKFRAFLEAQGGDPRAVEDFSLLPLAEEHPLRAEREGVVREVDAYKVGLAVLALGGGRKRKGEPIDHGVGVYLLKKPGDRVERGEALALVYHRRRGLEEALGHLREAYALGEEAHPAPLVLEAI

SEQ ID NO: 2 - DNA, 1272 bp, synthetic construct
  source 1..1272: mol_type = other DNA; note; note (original language) = 编码嘧啶核苷磷酸化酶的DNA序列
atgaacccggtggcgtttattcgcgaaaaacgcgaaggcaagaaacatcgccgcgaggatctggaagcgtttctgctgggctatctgcacgatgaagtgccggattatcaggtgagcgcgtggctgatggcggcgtttttacgcggcttagatccggaagaaaccctgtggctgaccgaaacgatggcccgcagcggtaaagtgctggatctgagcggtctgccgcatccggttgatcagcatagcagcggcggcgtgggcgataaagtgagcttagtggtgggcccgattctggcggcgagcggttgtacctttgcgaaaatgtcgggccgcaccctggcgcataccggtggtaacattgataaactggaaagcgtgccgggctggcgcggcgaaatgaccgaagcagaatttctggaacgcgcccgtcgcgttggtctggttattgcggcgcaaagcccggatttaacgccgttagatggcaaactgtatgcgctgcgcgatgtgaccgcgaccactgaatcagttccgctgattgcgagcagcattatgagcaagaaactggcggtgggcgcccgtagcattgtgttagatgttaaagtgggccgcggcgcgtttatgaaaaccctggaagaagcgcgtctgctggcgaaaacgatggtggcgattggccagggcgatggccgtcgtgttcgtgcgttattaaccagcatggaagcgcctctgggtcgtgcggttggcaatgcgattgaagtgcgtgaagcgattgaagcgctgaaaggcgaaggcccgggcgatttattagaagtggcgctggcgttagcggaagaagcgctgcgtcgtgaaggcttagatccggcgctggcgcgtaaagcgttagaaggtggcgcggcgctggaaaaatttcgcgcgtttctggaagcgcagggcggcgatccgcgtgcagttgaagattttagcctgctgccgctggcggaagaacatccgttacgtgcggaacgcgaaggcgtggttcgcgaagttgatgcgtataaagtgggcctggcggtgctggcgttaggcggtggtcgtaaacgtaaaggtgaaccgattgatcatggcgtgggcgtgtatctgctgaagaaaccgggcgatcgcgtggaacgcggcgaagcgttagcgttagtgtatcatcgccgccgcggcttagaagaagcgctgggtcatttacgcgaagcgtatgcgctgggcgaagaagcgcatccggcgcctctggttttagaagcgatttaa

SEQ ID NO: 3 - protein, 234 aa, Geobacillus stearothermophilus
MSVHIGAKEHEIADKILLPGDPLRAKYIAETFLEGATCYNQVRGMLGFTGTYKGHRISVQGTGMGVPSISIYITELMQSYNVQTLIRVGTCGAIQKDVKVRDVILAMTSSTDSQMNRMTFGGIDYAPTANFDLLKTAYEIGKEKGLQLKVGSVFTADMFYNENAQFEKLARYGVLAVEMETTALYTLAAKFGRKALSVLTVSDHILTGEETTAEERQTTFNEMIEVALETAIRQ